European Patent Application EP 4 357 460 A1, published April 24, 2024. Title: Fumonisin enzymatic degradation. Applicant: CONSEJO SUPERIOR DE INVESTIGACIONES CIENTIFICAS (CSIC). The sequence listing filed with the application follows.

SEQUENCE LISTING (4 sequences)

SEQ ID NO: 1 - protein, 448 aa, synthetic construct
MSTARLTPTSASTLKLLSVAVAALTLSACLSGGGGGGADGPNPLAIETSEGKVVGISNDGIRVFRGIPYAAPPVGDLRLAPPQPPASRSETLRLSEEFGNSCPQSDLTTGQQVGNEDCLYLNVYAPAEAEDLPVMVWIHGGAFVFGNGGGEYDPTRLVEQDVIVVTLNYRLGNLGFLAHPALESDAGNFALMDQQLALAWVKENITAFGGDPANVTIFGESAGGHSVMSHIVSPRAEEADLFQRAIVQSGSYAPFQMPKATAQFLGTSVANGLGCTDPETAASCLRSLPVSAFLAAQGSQSIPVVDPDDDLLPKSIQQALADGDFNSSLDIMIGSNQNEGTLFVALDEVGGDPIDGEAEYRERVAEFFQPYQASIPFDDDQIATDYLDFVDGEAKPFEAALSGIWTDFMFACNAYSQASTFAGASMNTFQYWFRDEDAPWTLVPPFAV

SEQ ID NO: 2 - protein, 575 aa, synthetic construct
MAHHHHHHVGTGSNDDDDKSPDPMSTARLTPTSASTLKLLSVAVAALTLSACLSGGGGGGADGPNPLAIETSEGKVVGISNDGIRVFRGIPYAAPPVGDLRLAPPQPPASRSETLRLSEEFGNSCPQSDLTTGQQVGNEDCLYLNVYAPAEAEDLPVMVWIHGGAFVFGNGGGEYDPTRLVEQDVIVVTLNYRLGNLGFLAHPALESDAGNFALMDQQLALAWVKENITAFGGDPANVTIFGESAGGHSVMSHIVSPRAEEADLFQRAIVQSGSYAPFQMPKATAQFLGTSVANGLGCTDPETAASCLRSLPVSAFLAAQGSQSIPVVDPDDDLLPKSIQQALADGDFNSSLDIMIGSNQNEGTLFVALDEVGGDPIDGEAEYRERVAEFFQPYQASIPFDDDQIATDYLDFVDGEAKPFEAALSGIWTDFMFACNAYSQASTFAGASMNTFQYWFRDEDAPWTLVPPFAVSFPLGATHAGEIPYVLYPQAIMEQRYTGDPDDLNSLAGEMVDYWTQFAKTGDPNTTDGVAAAWQQAATGNLMTLDVPNASNANTLGFLGYHHCSYWADPPLVLR

SEQ ID NO: 3 - protein, 539 aa, Sphingopyxis sp.
MKEHQCRGGRASPAAPATWLARISVSRGASAIAWTFMLGATAIPVAAQTDDPKLVRHTQSGAVEGVEGDVETFLGIPFAAPPVGDLRWRPPAPPRAWAGTRDGRRFAPDCIGNERLREGSRAAGTSEDCLYLNIWSPKQVGKGGLPVMIWVYGGGFSGGSGAVPYYDGSALAQKGVVVVTFNYRAGILGFLAHPALSKESPNGVSGNYGLLDMLAAFKWVQNNIREFGGDPNRVTVFGESAGASALGLLLTSPLSESAFNQAILQSPGLARPLATLSESEANGLELGADISALRRADAGLTKIAQSRIPMSRQFTKPRPMGPILDGYVLRTLDVDAFAKGAFRKIPVLVGGNADEGRAFTDRLPVKTVLEYRAYLTEQFGDEADAWERCYPANSDADVPAAVARLFGDSQFNNGIELLSAAFAKWRTPLWRYRFTGIPGAGRRPATHGDEIPYVFANLGPSSVSMFGSLEGGAGASDIKLATEMSAAWVSFAVHGVPDQGTKSHWPRFERRGEIMTFGSQVGSGEGLGVSPSKACQPSK

SEQ ID NO: 4 - DNA, 1635 bp, synthetic construct
  source 1..1635: mol_type = other DNA
atgctgctgagcggccgtaccttcgcgctggtgtttggtgcgccgctgctgggtgcgctggcggcgttcgcggtgccggttgcggcggcgagcggtcgtccgaccgcgaccgtggcggaaggtcgtgttgcgggcagcctggaggacggtgtgcgtgtttttaaaggtctgccgtatgcgctgccgccggtgggtgttcgtcgttggcgtccgccggctccgccggcgagctggcaaggtgcgcgtgaagcgcatgcgtttggtccggattgcgtgcaaccgccgtacccggcggacagcgtttattttgaaccgccgcgtccgaccagcgaggattgcctgaccctgaacgtttgggcgccgcgtagcgcggcgcgtgcgccggtgattgtttggattcacggtggcgcgctgcagcatggtggcagcgcgagcccgatgtatgacggtcgtgagtatgcgaaacgtggcatcgtgttcgttagcattaactaccgtctgggtatctttggttggctggcgcacccgggtctgagcgcggaagcgccggatcgtgtgagcggtaactatggtctgctggaccagattgcggcgctggagtgggttaagcgtaacattgcggcgtttggtggcgatccggcgaacgtgaccgcgatgggtgaaagcgcgggtgcgctgagcgttacctacctgctggcggcgccgcgtgcgaaaggtctgtttggccgtgcgatcgtgcaaagcaccaacatgcgtgcggttccgcgtctgcgtgacccggcgtatggtctgccgagcgcggaagcgatcggtgcggcgtttgcggagagcgtgggtgcgaagaacccggcggcgctgcgtgcgctggatgcggaggcgctgaccgcggcggcgctgcgcgcgcgctttgcggcgcagccgaccattgatggtgcgctgctgccggcgcagattgtggatgttttcgaccgtggtgaacaaatcaaagtgccggttctggcgggttttaacagcggcgaggtgcgcagccaacgtggtctggtgccgccggttccggcggatgcggcggcgtatgcggcgggtgcggcgcgtcgttatggtgacctggcgccggcgttcctgcgtctgtacccggcgagcgatatggaggaaagcctgatcgcggcgacccgtgacattgtttatggctgggcggtggaacgtctggttcgtcagcaaaccgtggcgggtgttccgagctacctgtacctgttcgatcactgctatgatgcggcgcgtgcgcgtaagctgtgcgcgtttcacgcgagcgagatcccgttcatgtttggtagcattggccgtgcggtgccgcaggcggcgaactggccggcggcgaccggtgatgatgaccgtcgtctggcgcgtcaaatggtggattattggagcagcttcgcggcgcgtggtatcccgagcgcggttggtgcgccggactggcgtccgtacggcgaggaagagtattttctggaactgggtgcgagcccggttctgcgtcgtgatccgatgccgggcatgttcgagtttcgtgaagagattatgcgtcgtcagcgtcaacgtggcgaacagtggttcgtgaacaccggtccggttgaccgtgag